European Patent Specification EP 2 983 686 B1, published May 29, 2024. Title: STABILIZED HUMAN IMMUNODEFICIENCY VIRUS (HIV) ENVELOPE (ENV) TRIMER VACCINES AND METHODS OF USING SAME. Applicant: BETH ISRAEL DEACONESS MEDICAL CENTER, INC. The sequence listing filed with the application follows.

SEQUENCE LISTING (32 sequences)

SEQ ID NO: 1 - protein, 712 aa, Artificial Sequence
  Synthetic Construct (mEnv)
MRVTGIRKNYQHLWRWGTMLLGILMICSAAGKLWVTVYYGVPVWKEATTTLFCASDAKAYDTEVHNVWATHACVPTDPNPQEVVLENVTENFNMWKNNMVEQMHEDIISLWDQSLKPCVKLTPLCVTLNCTDDVRNVTNNATNTNSSWGEPMEKGEIKNCSFNITTSIRNKVQKQYALFYKLDVVPIDNDSNNTNYRLISCNTSVITQACPKVSFEPIPIHYCAPAGFAILKCNDKKFNGTGPCTNVSTVQCTHGIRPVVSTQLLLNGSLAEEEVVIRSENFTNNAKTIMVQLNVSVEINCTRPNNNTRKSIHIGPGRAFYTAGDIIGDIRQAHCNISRANWNNTLRQIVEKLGKQFGNNKTIVFNHSSGGDPEIVMHSFNCGGEFFYCNSTKLFNSTWTWNNSTWNNTKRSNDTEEHITLPCRIKQIINMWQEVGKAMYAPPIRGQIRCSSNITGLLLTRDGGNDTSGTEIFRPGGGDMRDNWRSELYKYKVVKIEPLGVAPTKAKRRVVQSEKSAVGIGAVFLGFLGAAGSTMGAASMTLTVQARLLLSGIVQQQNNLLRAIEAQQHLLQLTVWGIKQLQARVLAVERYLKDQQLLGIWGCSGKLICTTTVPWNASWSNKSLDKIWNNMTWMEWEREINNYTSLIYTLIEESQNQQEKNEQELLELDKWASLWNWFDISNWLWGYIPEAPRDGQAYVRKDGEWVLLSTFL

SEQ ID NO: 2 - protein, 724 aa, Artificial Sequence
  Synthetic Construct (mEnv+)
MRVRGIQRNCQHLWRWGTLILGMLMICSAAGKLWVTVYYGVPVWKEATTTLFCASDAKAYDTEVHNVWATHACVPTDPNPQEVVLENVTENFNMWKNNMVEQMHEDIISLWDQSLKPCVKLTPLCVTLNCTDDVRNVTNNATNTNSSWGEPMEKGEIKNCSFNITTSIRNKVQKQYALFYKLDVVPIDNDSNNTNYRLISCNTSVITQACPKVSFEPIPIHYCAPAGFAILKCNDKKFNGTGPCTNVSTVQCTHGIRPVVSTQLLLNGSLAEEEVVIRSENFTNNAKTIMVQLNVSVEINCTRPNNNTRKSIHIGPGRAFYTAGDIIGDIRQAHCNISRANWNNTLRQIVEKLGKQFGNNKTIVFNHSSGGDPEIVMHSFNCGGEFFYCNSTKLFNSTWTWNNSTWNNTKRSNDTEEHITLPCRIKQIINMWQEVGKAMYAPPIRGQIRCSSNITGLLLTRDGGNDTSGTEIFRPGGGDMRDNWRSELYKYKVVKIEPLGVAPTKAKERVVQREERAVGIGAVFLGFLGAAGSTMGAASMTLTVQARLLLSGIVQQQNNLLRAIEAQQHLLQLTVWGIKQLQARVLAVERYLKDQQLLGIWGCSGKLICTTTVPWNASWSNKSLDKIWNNMTWMEWEREINNYTSLIYTLIEESQNQQEKNEQELLELDKWASLWNWFDISNWLWYIKSRIEGRGSGGYIPEAPRDGQAYVRKDGEWVLLSTFL

SEQ ID NO: 3 - protein, 708 aa, Artificial Sequence
  Synthetic Construct (cEnv)
MRVRGIQRNCQHLWRWGTLILGMLMICSAAENLWVGNMWVTVYYGVPVWTDAKTTLFCASDTKAYDREVHNVWATHACVPTDPNPQEIVLENVTENFNMWKNDMVDQMHEDIISLWDQSLKPCVKLTPLCVTLHCTNATFKNNVTNDMNKEIRNCSFNTTTEIRDKKQQGYALFYRPDIVLLKENRNNSNNSEYILINCNASTITQACPKVNFDPIPIHYCAPAGYAILKCNNKTFSGKGPCNNVSTVQCTHGIKPVVSTQLLLNGSLAEKEIIIRSENLTDNVKTIIVHLNKSVEIVCTRPNNNTRKSMRIGPGQTFYATGDIIGDIRQAYCNISGSKWNETLKRVKEKLQENYNNNKTIKFAPSSGGDLEITTHSFNCRGEFFYCNTTRLFNNNATEDETITLPCRIKQIINMWQGVGRAMYAPPIAGNITCKSNITGLLLVRDGGEDNKTEEIFRPGGGNMKDNWRSELYKYKVIELKPLGIAPTGAKERVVEREERAVGIGAVFLGFLGAAGSTMGAASLTLTVQARQLLSSIVQQQSNLLRAIEAQQHMLQLTVWGIKQLQTRVLAIERYLKDQQLLGIWGCSGKLICTTNVPWNSSWSNKSQTDIWNNMTWMEWDREISNYTDTIYRLLEDSQTQQEKNEKDLLALDSWKNLWSWFDISNWLWYIKSRIEGRGSGGYIPEAPRDGQAYVRKDGEWVLLSTFL

SEQ ID NO: 4 - protein, 684 aa, Artificial Sequence
  Synthetic Construct (mEnv2)
MRVRGIQRNWPQWWIWGILGFWMIIICRVMGNLWVTVYYGVPVWKEAKTTLFCASDAKAYEKEVHNVWATHACVPTDPNPQEMVLENVTENFNMWKNDMVDQMHEDIIRLWDQSLKPCVKLTPLCVTLECRNVRNVSSNGTYNIIHNETYKEMKNCSFNATTVVEDRKQKVHALFYRLDIVPLDENNSSEKSSENSSEYYRLINCNTSAITQACPKVSFDPIPIHYCAPAGYAILKCNNKTFNGTGPCNNVSTVQCTHGIKPVVSTQLLLNGSLAEEEIIIRSENLTNNAKTIIVHLNETVNITCTRPNNNTRKSIRIGPGQTFYATGDIIGDIRQAHCNLSRDGWNKTLQGVKKKLAEHFPNKTINFTSSSGGDLEITTHSFNCRGEFFYCNTSGLFNGTYMPNGTNSNSSSNITLPCRIKQIINMWQEVGRAMYAPPIAGNITCRSNITGLLLTRDGGSNNGVPNDTETFRPGGGDMRNNWRSELYKYKVVEVKPLGVAPTEAKRRVVESEKSAVGIGAVFLGILGAAGSTMGAASITLTVQARQLLSGIVQQQSNLLRAIEAQQHMLQLTVWGIKQLQTRVLAIERYLQDQQLLGLWGCSGKLICTTAVPWNTSWSNKSQTDIWDNMTWMQWDKEIGNYTGEIYRLLEESQNQQEKNEKDLLALDSWKNLWNWFDITNWLW

SEQ ID NO: 5 - protein, 678 aa, Artificial Sequence
  Synthetic Construct (mEnv3)
MRVKGIRKNYQHLWKWGTMLLGMLMICSAAEQLWVTVYYGVPVWRDAETTLFCASDAKAYEREVHNIWATHACVPTDPNPQEIVLENVTEEFNMWKNDMVEQMHTDIISLWDESLKPCVKLAPLCVTLNCTNANLNCTNDNCNRTVDKMREEIKNCSFNMTTELRDKKQKVYALFYKLDIVPIEKNSSEYRLINCNTSTITQACPKVTFEPIPIHYCTPAGFAILKCKDKKFNGTGPCKNVSTVQCTHGIKPVISTQLLLNGSLAEGEIIIRSENITNNAKTIIVQLNESVVINCTRPGNNTRKSVRIGPGQAFYATGEIIGDIRQAYCNISRAKWNNTLKQIVTKLKEQFKNKTIVFNQSSGGDPEITTHSFNCGGEFFYCNTTQLFNSTWNSNSTWNDTTGSVTEGNDTITLPCRIKQIVNMWQRVGQAMYAPPIEGNITCKSNITGLLLVRDGGNINRTNETFRPGGGNMKDNWRSELYKYKVVEIKPLGVAPTRAKRRVVESEKSAVGLGAVFLGFLGTAGSTMGAASLTLTVQARQVLSGIVQQQSNLLKAIEAQQHLLKLTVWGIKQLQARILAVERYLRDQQLLGIWGCSGKLICTTNVPWNSSWSNKSQEEIWNNMTWMQWDREISNYTDTIYRLLEDSQNQQEKNEQDLLALDKWASLWNWFSITNWLW

SEQ ID NO: 6 - protein, 685 aa, Artificial Sequence
  Synthetic Construct (Mosaic gp140 Env1)
MRVTGIRKNYQHLWRWGTMLLGILMICSAAGKLWVTVYYGVPVWKEATTTLFCASDAKAYDTEVHNVWATHACVPTDPNPQEVVLENVTENFNMWKNNMVEQMHEDIISLWDQSLKPCVKLTPLCVTLNCTDDVRNVTNNATNTNSSWGEPMEKGEIKNCSFNITTSIRNKVQKQYALFYKLDVVPIDNDSNNTNYRLISCNTSVITQACPKVSFEPIPIHYCAPAGFAILKCNDKKFNGTGPCTNVSTVQCTHGIRPVVSTQLLLNGSLAEEEVVIRSENFTNNAKTIMVQLNVSVEINCTRPNNNTRKSIHIGPGRAFYTAGDIIGDIRQAHCNISRANWNNTLRQIVEKLGKQFGNNKTIVFNHSSGGDPEIVMHSFNCGGEFFYCNSTKLFNSTWTWNNSTWNNTKRSNDTEEHITLPCRIKQIINMWQEVGKAMYAPPIRGQIRCSSNITGLLLTRDGGNDTSGTEIFRPGGGDMRDNWRSELYKYKVVKIEPLGVAPTKAKRRVVQSEKSAVGIGAVFLGFLGAAGSTMGAASMTLTVQARLLLSGIVQQQNNLLRAIEAQQHLLQLTVWGIKQLQARVLAVERYLKDQQLLGIWGCSGKLICTTTVPWNASWSNKSLDKIWNNMTWMEWEREINNYTSLIYTLIEESQNQQEKNEQELLELDKWASLWNWFDISNWLW

SEQ ID NO: 7 - protein, 1350 aa, Artificial Sequence
  Synthetic Construct (Mosaic gagpol1 v3)
MGARASVLSGGELDRWEKIRLRPGGKKKYRLKHIVWASRELERFAVNPGLLETSEGCRQILGQLQPSLQTGSEELRSLYNTVATLYCVHQRIEIKDTKEALEKIEEEQNKSKKKAQQAAADTGNSSQVSQNYPIVQNIQGQMVHQAISPRTLNAWVKVVEEKAFSPEVIPMFSALSEGATPQDLNTMLNTVGGHQAAMQMLKETINEEAAEWDRVHPVHAGPIAPGQMREPRGSDIAGTTSTLQEQIGWMTNNPPIPVGEIYKRWIILGLNKIVRMYSPVSILDIRQGPKEPFRDYVDRFYKTLRAEQASQDVKNWMTETLLVQNANPDCKTILKALGPAATLEEMMTACQGVGGPGHKARVLAEAMSQVTNSATIMMQRGNFRNQRKTVKCFNCGKEGHIAKNCRAPRKKGCWKCGKEGHQMKDCTERQANFLGKIWPSNKGRPGNFLQNRPEPTAPPEESFRFGEETTTPSQKQEPIDKEMYPLASLKSLFGNDPSSQMAPISPIETVPVKLKPGMDGPRVKQWPLTEEKIKALTAICEEMEKEGKITKIGPENPYNTPVFAIKKKDSTKWRKLVDFRELNKRTQDFWEVQLGIPHPAGLKKKKSVTVLAVGDAYFSVPLDEGFRKYTAFTIPSTNNETPGIRYQYNVLPQGWKGSPAIFQCSMTRILEPFRAKNPEIVIYQYMAALYVGSDLEIGQHRAKIEELREHLLKWGFTTPDKKHQKEPPFLWMGYELHPDKWTVQPIQLPEKDSWTVNDIQKLVGKLNWASQIYPGIKVRQLCKLLRGAKALTDIVPLTEEAELELAENREILKEPVHGVYYDPSKDLIAEIQKQGHDQWTYQIYQEPFKNLKTGKYAKMRTAHTNDVKQLTEAVQKIAMESIVIWGKTPKFRLPIQKETWETWWTDYWQATWIPEWEFVNTPPLVKLWYQLEKDPIAGVETFYVAGAANRETKLGKAGYVTDRGRQKIVSLTETTNQKTALQAIYLALQDSGSEVNIVTASQYALGIIQAQPDKSESELVNQIIEQLIKKERVYLSWVPAHKGIGGNEQVDKLVSSGIRKVLFLDGIDKAQEEHEKYHSNWRAMASDFNLPPVVAKEIVASCDQCQLKGEAMHGQVDCSPGIWQLACTHLEGKIILVAVHVASGYIEAEVIPAETGQETAYFILKLAGRWPVKVIHTANGSNFTSAAVKAACWWAGIQQEFGIPYNPQSQGVVASMNKELKKIIGQVRDQAEHLKTAVQMAVFIHNFKRKGGIGGYSAGERIIDIIATDIQTKELQKQIIKIQNFRVYYRDSRDPIWKGPAKLLWKGEGAVVIQDNSDIKVVPRRKVKIIKDYGKQMAGADCVAGRQDED

SEQ ID NO: 8 - protein, 857 aa, Artificial Sequence
  Synthetic Construct (Mosaic gp160 Env1)
MRVTGIRKNYQHLWRWGTMLLGILMICSAAGKLWVTVYYGVPVWKEATTTLFCASDAKAYDTEVHNVWATHACVPTDPNPQEVVLENVTENFNMWKNNMVEQMHEDIISLWDQSLKPCVKLTPLCVTLNCTDDVRNVTNNATNTNSSWGEPMEKGEIKNCSFNITTSIRNKVQKQYALFYKLDVVPIDNDSNNTNYRLISCNTSVITQACPKVSFEPIPIHYCAPAGFAILKCNDKKFNGTGPCTNVSTVQCTHGIRPVVSTQLLLNGSLAEEEVVIRSENFTNNAKTIMVQLNVSVEINCTRPNNNTRKSIHIGPGRAFYTAGDIIGDIRQAHCNISRANWNNTLRQIVEKLGKQFGNNKTIVFNHSSGGDPEIVMHSFNCGGEFFYCNSTKLFNSTWTWNNSTWNNTKRSNDTEEHITLPCRIKQIINMWQEVGKAMYAPPIRGQIRCSSNITGLLLTRDGGNDTSGTEIFRPGGGDMRDNWRSELYKYKVVKIEPLGVAPTKAKRRVVQREKRAVGIGAVFLGFLGAAGSTMGAASMTLTVQARLLLSGIVQQQNNLLRAIEAQQHLLQLTVWGIKQLQARVLAVERYLKDQQLLGIWGCSGKLICTTTVPWNASWSNKSLDKIWNNMTWMEWEREINNYTSLIYTLIEESQNQQEKNEQELLELDKWASLWNWFDISNWLWYIKIFIMIVGGLVGLRIVFAVLSIVNRVRQGYSPLSFQTRLPAPRGPDRPEGIEEEGGERDRDRSVRLVDGFLVLIWDDLQSLCLFSYHRLRDLLLIVELLGRRGWEALKYWWNLLQYWSQELKNSAISLLNATAVAVAEGTDRVIEALQRACRAILHIPRRIRQGLERLLL

SEQ ID NO: 9 - protein, 867 aa, Artificial Sequence
  Synthetic Construct (Mosaic gp160 Env2)
MRVRGIQRNWPQWWIWGILGFWMIIICRVMGNLWVTVYYGVPVWKEAKTTLFCASDAKAYEKEVHNVWATHACVPTDPNPQEMVLENVTENFNMWKNDMVDQMHEDIIRLWDQSLKPCVKLTPLCVTLECRNVRNVSSNGTYNIIHNETYKEMKNCSFNATTVVEDRKQKVHALFYRLDIVPLDENNSSEKSSENSSEYYRLINCNTSAITQACPKVSFDPIPIHYCAPAGYAILKCNNKTFNGTGPCNNVSTVQCTHGIKPVVSTQLLLNGSLAEEEIIIRSENLTNNAKTIIVHLNETVNITCTRPNNNTRKSIRIGPGQTFYATGDIIGDIRQAHCNLSRDGWNKTLQGVKKKLAEHFPNKTINFTSSSGGDLEITTHSFNCRGEFFYCNTSGLFNGTYMPNGTNSNSSSNITLPCRIKQIINMWQEVGRAMYAPPIAGNITCRSNITGLLLTRDGGSNNGVPNDTETFRPGGGDMRNNWRSELYKYKVVEVKPLGVAPTEAKRRVVEREKRAVGIGAVFLGILGAAGSTMGAASITLTVQARQLLSGIVQQQSNLLRAIEAQQHMLQLTVWGIKQLQTRVLAIERYLQDQQLLGLWGCSGKLICTTAVPWNTSWSNKSQTDIWDNMTWMQWDKEIGNYTGEIYRLLEESQNQQEKNEKDLLALDSWKNLWNWFDITNWLWYIKIFIMIVGGLIGLRIILGVLSIVRRVRQGYSPLSFQTLTPNPRGLDRLGRIEEEGGEQDRDRSIRLVNGFLALAWDDLRSLCLFSYHQLRDFILIVARAVELLGRSSLRGLQRGWEALKYLGNLVQYWGLELKKGAISLLDTIAIAVAEGTDRIIELIQSICRAIRNIPRRIRQGFEASLL

SEQ ID NO: 10 - protein, 500 aa, Artificial Sequence
  Synthetic Construct (Mosaic gag1)
MGARASVLSGGELDRWEKIRLRPGGKKKYRLKHIVWASRELERFAVNPGLLETSEGCRQILGQLQPSLQTGSEELRSLYNTVATLYCVHQRIEIKDTKEALEKIEEEQNKSKKKAQQAAADTGNSSQVSQNYPIVQNIQGQMVHQAISPRTLNAWVKVVEEKAFSPEVIPMFSALSEGATPQDLNTMLNTVGGHQAAMQMLKETINEEAAEWDRVHPVHAGPIAPGQMREPRGSDIAGTTSTLQEQIGWMTNNPPIPVGEIYKRWIILGLNKIVRMYSPVSILDIRQGPKEPFRDYVDRFYKTLRAEQASQDVKNWMTETLLVQNANPDCKTILKALGPAATLEEMMTACQGVGGPGHKARVLAEAMSQVTNSATIMMQRGNFRNQRKTVKCFNCGKEGHIAKNCRAPRKKGCWKCGKEGHQMKDCTERQANFLGKIWPSNKGRPGNFLQNRPEPTAPPEESFRFGEETTTPSQKQEPIDKEMYPLASLKSLFGNDPSSQ

SEQ ID NO: 11 - protein, 491 aa, Artificial Sequence
  Synthetic Construct (Mosaic gag2)
MGARASILRGGKLDKWEKIRLRPGGKKHYMLKHLVWASRELERFALNPGLLETSEGCKQIIKQLQPALQTGTEELRSLFNTVATLYCVHAEIEVRDTKEALDKIEEEQNKSQQKTQQAKEADGKVSQNYPIVQNLQGQMVHQPISPRTLNAWVKVIEEKAFSPEVIPMFTALSEGATPQDLNTMLNTVGGHQAAMQMLKDTINEEAAEWDRLHPVHAGPVAPGQMREPRGSDIAGTTSNLQEQIAWMTSNPPIPVGDIYKRWIILGLNKIVRMYSPTSILDIKQGPKEPFRDYVDRFFKTLRAEQATQDVKNWMTDTLLVQNANPDCKTILRALGPGATLEEMMTACQGVGGPSHKARVLAEAMSQTNSTILMQRSNFKGSKRIVKCFNCGKEGHIARNCRAPRKKGCWKCGKEGHQMKDCTERQANFLGKIWPSHKGRPGNFLQSRPEPTAPPAESFRFEETTPAPKQEPKDREPLTSLRSLFGSDPLSQ

SEQ ID NO: 12 - protein, 999 aa, Artificial Sequence
  Synthetic Construct (Mosaic pol1)
FFRENLAFQQGEAREFPSEQTRANSPTSRELQVRGDNPHSEAGAERQGTLNFPQITLWQRPLVSIKVGGQIREALLDTGADDTVLEDINLPGKWKPKMIGGIGGFIKVRQYDQILIEICGKKAIGTVLVGPTPVNIIGRNMLTQLGCTLNFPISPIETVPVKLKPGMDGPRVKQWPLTEEKIKALTAICEEMEKEGKITKIGPENPYNTPVFAIKKKDSTKWRKLVDFRELNKRTQDFWEVQLGIPHPAGLKKKKSVTVLDVGDAYFSVPLDEGFRKYTAFTIPSTNNETPGIRYQYNVLPQGWKGSPAIFQCSMTRILEPFRAKNPEIVIYQYMDDLYVGSDLEIGQHRAKIEELREHLLKWGFTTPDKKHQKEPPFLWMGYELHPDKWTVQPIQLPEKDSWTVNDIQKLVGKLNWASQIYPGIKVRQLCKLLRGAKALTDIVPLTEEAELELAENREILKEPVHGVYYDPSKDLIAEIQKQGHDQWTYQIYQEPFKNLKTGKYAKMRTAHTNDVKQLTEAVQKIAMESIVIWGKTPKFRLPIQKETWETWWTDYWQATWIPEWEFVNTPPLVKLWYQLEKDPIAGVETFYVDGAANRETKLGKAGYVTDRGRQKIVSLTETTNQKTELQAIYLALQDSGSEVNIVTDSQYALGIIQAQPDKSESELVNQIIEQLIKKERVYLSWVPAHKGIGGNEQVDKLVSSGIRKVLFLDGIDKAQEEHEKYHSNWRAMASDFNLPPVVAKEIVASCDQCQLKGEAMHGQVDCSPGIWQLDCTHLEGKIILVAVHVASGYIEAEVIPAETGQETAYFILKLAGRWPVKVIHTDNGSNFTSAAVKAACWWAGIQQEFGIPYNPQSQGVVESMNKELKKIIGQVRDQAEHLKTAVQMAVFIHNFKRKGGIGGYSAGERIIDIIATDIQTKELQKQIIKIQNFRVYYRDSRDPIWKGPAKLLWKGEGAVVIQDNSDIKVVPRRKVKIIKDYGKQMAGADCVAGRQDED

SEQ ID NO: 13 - protein, 1003 aa, Artificial Sequence
  Synthetic Construct (Mosaic pol2)
FFRENLAFPQGKAREFSSEQTRANSPTRRELQVWGRDNNSLSEAGADRQGTVSFSFPQITLWQRPLVTIKIGGQLKEALLDTGADDTVLEEMNLPGRWKPKMIGGIGGFIKVRQYDQIPIEICGHKAIGTVLVGPTPVNIIGRNLLTQIGCTLNFPISPIETVPVKLKPGMDGPKVKQWPLTEEKIKALVEICTEMEKEGKISKIGPENPYNTPIFAIKKKDSTKWRKLVDFRELNKRTQDFWEVQLGIPHPAGLKKKKSVTVLDVGDAYFSVPLDEDFRKYTAFTIPSINNETPGIRYQYNVLPQGWKGSPAIFQSSMTKILEPFRKQNPDIVIYQYMDDLYVGSDLEIGQHRTKIEELRQHLLRWGFTTPDKKHQKEPPFLWMGYELHPDKWTVQPIVLPEKDSWTVNDIQKLVGKLNWASQIYAGIKVKQLCKLLRGTKALTEVVPLTEEAELELAENREILKEPVHGVYYDPSKDLIAEIQKQGQGQWTYQIYQEPFKNLKTGKYARMRGAHTNDVKQLTEAVQKIATESIVIWGKTPKFKLPIQKETWEAWWTEYWQATWIPEWEFVNTPPLVKLWYQLEKEPIVGAETFYVDGAANRETKLGKAGYVTDRGRQKVVSLTDTTNQKTELQAIHLALQDSGLEVNIVTDSQYALGIIQAQPDKSESELVSQIIEQLIKKEKVYLAWVPAHKGIGGNEQVDKLVSRGIRKVLFLDGIDKAQEEHEKYHSNWRAMASEFNLPPIVAKEIVASCDKCQLKGEAIHGQVDCSPGIWQLDCTHLEGKVILVAVHVASGYIEAEVIPAETGQETAYFLLKLAGRWPVKTIHTDNGSNFTSATVKAACWWAGIKQEFGIPYNPQSQGVVESINKELKKIIGQVRDQAEHLKTAVQMAVFIHNFKRKGGIGEYSAGERIVDIIASDIQTKELQKQITKIQNFRVYYRDSRDPLWKGPAKLLWKGEGAVVIQDNSDIKVVPRRKAKIIRDYGKQMAGDDCVASRQDED

SEQ ID NO: 14 - protein, 206 aa, Artificial Sequence
  Synthetic Construct (Mosaic nef1)
MGGKWSKSSVVGWPAIRERMRRAEPAADGVGAVSRDLEKHGAITSSNTAANNADCAWLEAQEEEEVGFPVRPQVPLRPMTYKGALDLSHFLKEKGGLEGLIYSQKRQDILDLWVYHTQGYFPDWQNYTPGPGIRYPLTFGWCFKLVPVEPEKIEEANEGENNSLLHPMSQHGMDDPEKEVLMWKFDSRLAFHHMARELHPEYYKDC

SEQ ID NO: 15 - protein, 206 aa, Artificial Sequence
  Synthetic Construct (Mosaic nef2)
MGGKWSKSSIVGWPAVRERIRRAEPAAEGVGAASQDLDKYGALTSSNTAATNADCAWLEAQEDEEVGFPVKPQVPLRPMTYKAAFDLSFFLKEKGGLDGLIYSKKRQEILDLWVYNTQGFFPDWQNYTPGPGVRYPLTFGWCFKLVPVDPREVEEANKGENNCLLHPMNLHGMDDPEREVLVWRFDSRLAFHHMAREKHPEYYKNC

SEQ ID NO: 16 - protein, 850 aa, Artificial Sequence
  Synthetic Construct (Mosaic pol1)
MAPISPIETVPVKLKPGMDGPRVKQWPLTEEKIKALTAICEEMEKEGKITKIGPENPYNTPVFAIKKKDSTKWRKLVDFRELNKRTQDFWEVQLGIPHPAGLKKKKSVTVLAVGDAYFSVPLDEGFRKYTAFTIPSTNNETPGIRYQYNVLPQGWKGSPAIFQCSMTRILEPFRAKNPEIVIYQYMAALYVGSDLEIGQHRAKIEELREHLLKWGFTTPDKKHQKEPPFLWMGYELHPDKWTVQPIQLPEKDSWTVNDIQKLVGKLNWASQIYPGIKVRQLCKLLRGAKALTDIVPLTEEAELELAENREILKEPVHGVYYDPSKDLIAEIQKQGHDQWTYQIYQEPFKNLKTGKYAKMRTAHTNDVKQLTEAVQKIAMESIVIWGKTPKFRLPIQKETWETWWTDYWQATWIPEWEFVNTPPLVKLWYQLEKDPIAGVETFYVAGAANRETKLGKAGYVTDRGRQKIVSLTETTNQKTALQAIYLALQDSGSEVNIVTASQYALGIIQAQPDKSESELVNQIIEQLIKKERVYLSWVPAHKGIGGNEQVDKLVSSGIRKVLFLDGIDKAQEEHEKYHSNWRAMASDFNLPPVVAKEIVASCDQCQLKGEAMHGQVDCSPGIWQLACTHLEGKIILVAVHVASGYIEAEVIPAETGQETAYFILKLAGRWPVKVIHTANGSNFTSAAVKAACWWAGIQQEFGIPYNPQSQGVVASMNKELKKIIGQVRDQAEHLKTAVQMAVFIHNFKRKGGIGGYSAGERIIDIIATDIQTKELQKQIIKIQNFRVYYRDSRDPIWKGPAKLLWKGEGAVVIQDNSDIKVVPRRKVKIIKDYGKQMAGADCVAGRQDED

SEQ ID NO: 17 - protein, 850 aa, Artificial Sequence
  Synthetic Construct (Mosaic pol1)
MAPISPIETVPVKLKPGMDGPKVKQWPLTEEKIKALVEICTEMEKEGKISKIGPENPYNTPIFAIKKKDSTKWRKLVDFRELNKRTQDFWEVQLGIPHPAGLKKKKSVTVLAVGDAYFSVPLDEDFRKYTAFTIPSINNETPGIRYQYNVLPQGWKGSPAIFQSSMTKILEPFRKQNPDIVIYQYMAALYVGSDLEIGQHRTKIEELRQHLLRWGFTTPDKKHQKEPPFLWMGYELHPDKWTVQPIVLPEKDSWTVNDIQKLVGKLNWASQIYAGIKVKQLCKLLRGTKALTEVVPLTEEAELELAENREILKEPVHGVYYDPSKDLIAEIQKQGQGQWTYQIYQEPFKNLKTGKYARMRGAHTNDVKQLTEAVQKIATESIVIWGKTPKFKLPIQKETWEAWWTEYWQATWIPEWEFVNTPPLVKLWYQLEKEPIVGAETFYVAGAANRETKLGKAGYVTDRGRQKVVSLTDTTNQKTALQAIHLALQDSGLEVNIVTASQYALGIIQAQPDKSESELVSQIIEQLIKKEKVYLAWVPAHKGIGGNEQVDKLVSRGIRKVLFLDGIDKAQEEHEKYHSNWRAMASEFNLPPIVAKEIVASCDKCQLKGEAIHGQVDCSPGIWQLACTHLEGKVILVAVHVASGYIEAEVIPAETGQETAYFLLKLAGRWPVKTIHTANGSNFTSATVKAACWWAGIKQEFGIPYNPQSQGVVASINKELKKIIGQVRDQAEHLKTAVQMAVFIHNFKRKGGIGEYSAGERIVDIIASDIQTKELQKQITKIQNFRVYYRDSRDPLWKGPAKLLWKGEGAVVIQDNSDIKVVPRRKAKIIRDYGKQMAGDDCVASRQDED

SEQ ID NO: 18 - protein, 851 aa, Artificial Sequence
  Synthetic Construct (Mos3 pol v3)
MAPISPIDTVPVTLKPGMDGPKIKQWPLTEEKIKALTEICTEMEKEGKISRIGPENPYNTPVFAIKKKNSTRWRKLVDFRELNKKTQDFWEVQLGIPHPAGLKKKRSVTVLAVGDAYFSVPLDKDFRKYTAFTIPSVNNETPGVRYQYNVLPQGWKGSPAIFQCSMTKILEPFRAQNPEIVIYQYVAALYVGSDLEIEQHRTKIEELRAHLLSWGFTTPDKKHQREPPFLWMGYELHPDRWTVQPIELPEKESWTVNDIQKLVGKLNWASQIYPGIKVKQLCRLLRGAKALTEVIPLTKEAELELAENREILREPVHGVYYDPSKDLVAEIQKQGQDQWTYQIYQEPYKNLKTGKYARKRSAHTNDVRQLTEAVQKIALESIVIWGKIPKFRLPIQRETWETWWTEYWQATWIPDWEFVNTPPLVKLWYQLEKEPIAGAETFYVAGASNRETKIGKAGYVTDKGRQKVVSLTETTNQKAALQAIQLALQDSGPEVNIVTASQYVLGIIQAQPDRSESELVNQIIEELIKKEKVYLSWVPAHKGIGGNEQVDKLVSAGIRKILFLDGIDKAQEEHERYHSNWRTMASDFNLPPIVAKEIVANCDKCQLKGEAMHGQVDCSPGMWQLACTHLEGKIIIVAVHVASGYMEAEVIPAETGQETAYYILKLAGRWPVKVVHTANGSNFTSTTVKAACWWANVTQEFGIPYNPQSQGVIASMNKELKKIIGQVREQAEHLKTAVQMAVLIHNFKRRGGIGGYSAGERIVDIIATDIQTRELQKQIIKIQNFRVYFRDSRDPVWKGPAKLLWKGEGAVVIQDNSEIKVVPRRKVKIIRDYGKQMAGDDCVAGRQDEDQ

SEQ ID NO: 19 - protein, 508 aa, Artificial Sequence
  Synthetic Construct (Mos3 gag)
MGARASVLSGGKLDAWEKIRLRPGGKKKYKLKHIVWASRELDRFALNPGLLETAEGCQQIIEQLQPALQTGSEELKSLYNTVAVLYCVHQRIDVKDTKEALDKIEEIQNKSKQKTQQAAADTGSSSKVSQNYPIVQNAQGQMVHQALSPRTLNAWVKVVEEKGFNPEVIPMFSALAEGATPQDLNMMLNIVGGHQAAMQILKDTINEEAADWDRLHPVHAGPIPPGQMREPRGSDIAGTTSTPQEQIGWMTSNPPVPVGEIYKRWIIMGLNKIVRMYSPVSILDIKQGPKESFRDYVDRFFKVLRAEQATQEVKNWMTETLLIQNANPDCKSILRALGPGASLEEMMTACQGVGGPSHKARILAEAMSQANNTNIMMQRGNFKGQKRIKCFNCGKEGHLARNCRAPRKRGCWKCGREGHQMKDCNERQANFLGKIWPSSKGRPGNFPQSRPEPTAPLEPTAPPAEPTAPPAESFGFGEEITPSPKQEQKDREPLTSLKSLFGSDPLLQ

SEQ ID NO: 20 - protein, 206 aa, Artificial Sequence
  Synthetic Construct ((Mos1 nef) (G to A to delete myristylation site))
MAGKWSKSSVVGWPAIRERMRRAEPAADGVGAVSRDLEKHGAITSSNTAANNADCAWLEAQEEEEVGFPVRPQVPLRPMTYKGALDLSHFLKEKGGLEGLIYSQKRQDILDLWVYHTQGYFPDWQNYTPGPGIRYPLTFGWCFKLVPVEPEKIEEANEGENNSLLHPMSQHGMDDPEKEVLMWKFDSRLAFHHMARELHPEYYKDC

SEQ ID NO: 21 - protein, 206 aa, Artificial Sequence
  Synthetic Construct ((Mos2 nef) (G to A to delete myristylation))
MAGKWSKSSIVGWPAVRERIRRAEPAAEGVGAASQDLDKYGALTSSNTAATNADCAWLEAQEDEEVGFPVKPQVPLRPMTYKAAFDLSFFLKEKGGLDGLIYSKKRQEILDLWVYNTQGFFPDWQNYTPGPGVRYPLTFGWCFKLVPVDPREVEEANKGENNCLLHPMNLHGMDDPEREVLVWRFDSRLAFHHMAREKHPEYYKNC

SEQ ID NO: 22 - protein, 208 aa, Artificial Sequence
  Synthetic Construct (Mos3 nef)
MAGKWSKRSVVGWPAVRERMRRTEPAAEGVGAVSQDLDKHGALTSSNTAHNNADCAWLQAQEEEEEVGFPVRPQVPVRPMTYKAAVDLSHFLKEKGGLEGLIHSQKRQEILDLWVYHTQGFFPDWHNYTPGPGTRFPLTFGWCYKLVPVDPKEVEEANEGENNCLLHPMSQHGMEDEDREVLKWKFDSSLARRHMARELHPEFYKDCL

SEQ ID NO: 23 - protein, 705 aa, Artificial Sequence
  Synthetic Construct (Mosaic gagnef1)
MGARASVLSGGELDRWEKIRLRPGGKKKYRLKHIVWASRELERFAVNPGLLETSEGCRQILGQLQPSLQTGSEELRSLYNTVATLYCVHQRIEIKDTKEALEKIEEEQNKSKKKAQQAAADTGNSSQVSQNYPIVQNIQGQMVHQAISPRTLNAWVKVVEEKAFSPEVIPMFSALSEGATPQDLNTMLNTVGGHQAAMQMLKETINEEAAEWDRVHPVHAGPIAPGQMREPRGSDIAGTTSTLQEQIGWMTNNPPIPVGEIYKRWIILGLNKIVRMYSPVSILDIRQGPKEPFRDYVDRFYKTLRAEQASQDVKNWMTETLLVQNANPDCKTILKALGPAATLEEMMTACQGVGGPGHKARVLAEAMSQVTNSATIMMQRGNFRNQRKTVKCFNCGKEGHIAKNCRAPRKKGCWKCGKEGHQMKDCTERQANFLGKIWPSNKGRPGNFLQNRPEPTAPPEESFRFGEETTTPSQKQEPIDKEMYPLASLKSLFGNDPSSQAGKWSKSSVVGWPAIRERMRRAEPAADGVGAVSRDLEKHGAITSSNTAANNADCAWLEAQEEEEVGFPVRPQVPLRPMTYKGALDLSHFLKEKGGLEGLIYSQKRQDILDLWVYHTQGYFPDWQNYTPGPGIRYPLTFGWCFKLVPVEPEKIEEANEGENNSLLHPMSQHGMDDPEKEVLMWKFDSRLAFHHMARELHPEYYKDC

SEQ ID NO: 24 - protein, 696 aa, Artificial Sequence
  Synthetic Construct (Mosaic gagnef2)
MGARASILRGGKLDKWEKIRLRPGGKKHYMLKHLVWASRELERFALNPGLLETSEGCKQIIKQLQPALQTGTEELRSLFNTVATLYCVHAEIEVRDTKEALDKIEEEQNKSQQKTQQAKEADGKVSQNYPIVQNLQGQMVHQPISPRTLNAWVKVIEEKAFSPEVIPMFTALSEGATPQDLNTMLNTVGGHQAAMQMLKDTINEEAAEWDRLHPVHAGPVAPGQMREPRGSDIAGTTSNLQEQIAWMTSNPPIPVGDIYKRWIILGLNKIVRMYSPTSILDIKQGPKEPFRDYVDRFFKTLRAEQATQDVKNWMTDTLLVQNANPDCKTILRALGPGATLEEMMTACQGVGGPSHKARVLAEAMSQTNSTILMQRSNFKGSKRIVKCFNCGKEGHIARNCRAPRKKGCWKCGKEGHQMKDCTERQANFLGKIWPSHKGRPGNFLQSRPEPTAPPAESFRFEETTPAPKQEPKDREPLTSLRSLFGSDPLSQAGKWSKSSIVGWPAVRERIRRAEPAAEGVGAASQDLDKYGALTSSNTAATNADCAWLEAQEDEEVGFPVKPQVPLRPMTYKAAFDLSFFLKEKGGLDGLIYSKKRQEILDLWVYNTQGFFPDWQNYTPGPGVRYPLTFGWCFKLVPVDPREVEEANKGENNCLLHPMNLHGMDDPEREVLVWRFDSRLAFHHMAREKHPEYYKNC

SEQ ID NO: 25 - protein, 1341 aa, Artificial Sequence
  Synthetic Construct (Mosaic gag pol2 v3)
MGARASILRGGKLDKWEKIRLRPGGKKHYMLKHLVWASRELERFALNPGLLETSEGCKQIIKQLQPALQTGTEELRSLFNTVATLYCVHAEIEVRDTKEALDKIEEEQNKSQQKTQQAKEADGKVSQNYPIVQNLQGQMVHQPISPRTLNAWVKVIEEKAFSPEVIPMFTALSEGATPQDLNTMLNTVGGHQAAMQMLKDTINEEAAEWDRLHPVHAGPVAPGQMREPRGSDIAGTTSNLQEQIAWMTSNPPIPVGDIYKRWIILGLNKIVRMYSPTSILDIKQGPKEPFRDYVDRFFKTLRAEQATQDVKNWMTDTLLVQNANPDCKTILRALGPGATLEEMMTACQGVGGPSHKARVLAEAMSQTNSTILMQRSNFKGSKRIVKCFNCGKEGHIARNCRAPRKKGCWKCGKEGHQMKDCTERQANFLGKIWPSHKGRPGNFLQSRPEPTAPPAESFRFEETTPAPKQEPKDREPLTSLRSLFGSDPLSQMAPISPIETVPVKLKPGMDGPKVKQWPLTEEKIKALVEICTEMEKEGKISKIGPENPYNTPIFAIKKKDSTKWRKLVDFRELNKRTQDFWEVQLGIPHPAGLKKKKSVTVLAVGDAYFSVPLDEDFRKYTAFTIPSINNETPGIRYQYNVLPQGWKGSPAIFQSSMTKILEPFRKQNPDIVIYQYMAALYVGSDLEIGQHRTKIEELRQHLLRWGFTTPDKKHQKEPPFLWMGYELHPDKWTVQPIVLPEKDSWTVNDIQKLVGKLNWASQIYAGIKVKQLCKLLRGTKALTEVVPLTEEAELELAENREILKEPVHGVYYDPSKDLIAEIQKQGQGQWTYQIYQEPFKNLKTGKYARMRGAHTNDVKQLTEAVQKIATESIVIWGKTPKFKLPIQKETWEAWWTEYWQATWIPEWEFVNTPPLVKLWYQLEKEPIVGAETFYVAGAANRETKLGKAGYVTDRGRQKVVSLTDTTNQKTALQAIHLALQDSGLEVNIVTASQYALGIIQAQPDKSESELVSQIIEQLIKKEKVYLAWVPAHKGIGGNEQVDKLVSRGIRKVLFLDGIDKAQEEHEKYHSNWRAMASEFNLPPIVAKEIVASCDKCQLKGEAIHGQVDCSPGIWQLACTHLEGKVILVAVHVASGYIEAEVIPAETGQETAYFLLKLAGRWPVKTIHTANGSNFTSATVKAACWWAGIKQEFGIPYNPQSQGVVASINKELKKIIGQVRDQAEHLKTAVQMAVFIHNFKRKGGIGEYSAGERIVDIIASDIQTKELQKQITKIQNFRVYYRDSRDPLWKGPAKLLWKGEGAVVIQDNSDIKVVPRRKAKIIRDYGKQMAGDDCVASRQDED

SEQ ID NO: 26 - protein, 1359 aa, Artificial Sequence
  Synthetic Construct (Mos3 gag-pol v3)
MGARASVLSGGKLDAWEKIRLRPGGKKKYKLKHIVWASRELDRFALNPGLLETAEGCQQIIEQLQPALQTGSEELKSLYNTVAVLYCVHQRIDVKDTKEALDKIEEIQNKSKQKTQQAAADTGSSSKVSQNYPIVQNAQGQMVHQALSPRTLNAWVKVVEEKGFNPEVIPMFSALAEGATPQDLNMMLNIVGGHQAAMQILKDTINEEAADWDRLHPVHAGPIPPGQMREPRGSDIAGTTSTPQEQIGWMTSNPPVPVGEIYKRWIIMGLNKIVRMYSPVSILDIKQGPKESFRDYVDRFFKVLRAEQATQEVKNWMTETLLIQNANPDCKSILRALGPGASLEEMMTACQGVGGPSHKARILAEAMSQANNTNIMMQRGNFKGQKRIKCFNCGKEGHLARNCRAPRKRGCWKCGREGHQMKDCNERQANFLGKIWPSSKGRPGNFPQSRPEPTAPLEPTAPPAEPTAPPAESFGFGEEITPSPKQEQKDREPLTSLKSLFGSDPLLQMAPISPIDTVPVTLKPGMDGPKIKQWPLTEEKIKALTEICTEMEKEGKISRIGPENPYNTPVFAIKKKNSTRWRKLVDFRELNKKTQDFWEVQLGIPHPAGLKKKRSVTVLAVGDAYFSVPLDKDFRKYTAFTIPSVNNETPGVRYQYNVLPQGWKGSPAIFQCSMTKILEPFRAQNPEIVIYQYVAALYVGSDLEIEQHRTKIEELRAHLLSWGFTTPDKKHQREPPFLWMGYELHPDRWTVQPIELPEKESWTVNDIQKLVGKLNWASQIYPGIKVKQLCRLLRGAKALTEVIPLTKEAELELAENREILREPVHGVYYDPSKDLVAEIQKQGQDQWTYQIYQEPYKNLKTGKYARKRSAHTNDVRQLTEAVQKIALESIVIWGKIPKFRLPIQRETWETWWTEYWQATWIPDWEFVNTPPLVKLWYQLEKEPIAGAETFYVAGASNRETKIGKAGYVTDKGRQKVVSLTETTNQKAALQAIQLALQDSGPEVNIVTASQYVLGIIQAQPDRSESELVNQIIEELIKKEKVYLSWVPAHKGIGGNEQVDKLVSAGIRKILFLDGIDKAQEEHERYHSNWRTMASDFNLPPIVAKEIVANCDKCQLKGEAMHGQVDCSPGMWQLACTHLEGKIIIVAVHVASGYMEAEVIPAETGQETAYYILKLAGRWPVKVVHTANGSNFTSTTVKAACWWANVTQEFGIPYNPQSQGVIASMNKELKKIIGQVREQAEHLKTAVQMAVLIHNFKRRGGIGGYSAGERIVDIIATDIQTRELQKQIIKIQNFRVYFRDSRDPVWKGPAKLLWKGEGAVVIQDNSEIKVVPRRKVKIIRDYGKQMAGDDCVAGRQDEDQ

SEQ ID NO: 27 - protein, 1497 aa, Artificial Sequence
  Synthetic Construct (Mosaic gagpol1 v4)
MGARASVLSGGELDRWEKIRLRPGGKKKYRLKHIVWASRELERFAVNPGLLETSEGCRQILGQLQPSLQTGSEELRSLYNTVATLYCVHQRIEIKDTKEALEKIEEEQNKSKKKAQQAAADTGNSSQVSQNYPIVQNIQGQMVHQAISPRTLNAWVKVVEEKAFSPEVIPMFSALSEGATPQDLNTMLNTVGGHQAAMQMLKETINEEAAEWDRVHPVHAGPIAPGQMREPRGSDIAGTTSTLQEQIGWMTNNPPIPVGEIYKRWIILGLNKIVRMYSPVSILDIRQGPKEPFRDYVDRFYKTLRAEQASQDVKNWMTETLLVQNANPDCKTILKALGPAATLEEMMTACQGVGGPGHKARVLAEAMSQVTNSATIMMQRGNFRNQRKTVKCFNCGKEGHIAKNCRAPRKKGCWKCGKEGHQMKDCTERQANFLGKIWPSNKGRPGNFLQNRPEPTAPPEESFRFGEETTTPSQKQEPIDKEMYPLASLKSLFGNDPSSQRENLAFQQGEAREFPSEQTRANSPTSRELQVRGDNPHSEAGAERQGTLNFPQITLWQRPLVSIKVGGQIREALLATGADDTVLEDINLPGKWKPKMIGGIGGFIKVGQYDQILIEICGKKAIGTVLVGPTPVNIIGRNMLTQLGCTLNFPISPIETVPVKLKPGMDGPRVKQWPLTEEKIKALTAICEEMEKEGKITKIGPENPYNTPVFAIKKKDSTKWRKLVDFRELNKRTQDFWEVQLGIPHPAGLKKKKSVTVLDVGDAYFSVPLDEGFRKYTAFTIPSTNNETPGIRYQYNVLPQGWKGSPAIFQCSMTRILEPFRAKNPEIVIYQYMDHLYVGSDLEIGQHRAKIEELREHLLKWGFTTPDKKHQKEPPFLWMGYELHPDKWTVQPIQLPEKDSWTVNDIQKLVGKLNWASQIYPGIKVRQLCKLLRGAKALTDIVPLTEEAELELAENREILKEPVHGVYYDPSKDLIAEIQKQGHDQWTYQIYQEPFKNLKTGKYAKMRTAHTNDVKQLTEAVQKIAMESIVIWGKTPKFRLPIQKETWETWWTDYWQATWIPEWEFVNTPPLVKLWYQLEKDPIAGVETFYVDGAANRETKLGKAGYVTDRGRQKIVSLTETTNQKTELQAIYLALQDSGSEVNIVTDSQYALGIIQAQPDKSESELVNQIIEQLIKKERVYLSWVPAHKGIGGNEQVDKLVSSGIRKVLFLDGIDKAQEEHEKYHSNWRAMASDFNLPPVVAKEIVASCDQCQLKGEAMHGQVDCSPGIWQLACTHLEGKIILVAVHVASGYIEAEVIPAETGQETAYFILKLAGRWPVKVIHTDNGSNFTSAAVKAACWWAGIQQEFGIPYNPQSQGVVESMNKELKKIIGQVRDQAEHLKTAVQMAVFIHNFKRKGGIGGYSAGERIIDIIATDIQTKELQKQIIKIQNFRVYYRDSRDPIWKGPAKLLWKGEGAVVIQDNSDIKVVPRRKVKIIKDYGKQMAGADCVAGRQDED

SEQ ID NO: 28 - protein, 1492 aa, Artificial Sequence
  Synthetic Construct (Mosaic gagpol2 v4)
MGARASILRGGKLDKWEKIRLRPGGKKHYMLKHLVWASRELERFALNPGLLETSEGCKQIIKQLQPALQTGTEELRSLFNTVATLYCVHAEIEVRDTKEALDKIEEEQNKSQQKTQQAKEADGKVSQNYPIVQNLQGQMVHQPISPRTLNAWVKVIEEKAFSPEVIPMFTALSEGATPQDLNTMLNTVGGHQAAMQMLKDTINEEAAEWDRLHPVHAGPVAPGQMREPRGSDIAGTTSNLQEQIAWMTSNPPIPVGDIYKRWIILGLNKIVRMYSPTSILDIKQGPKEPFRDYVDRFFKTLRAEQATQDVKNWMTDTLLVQNANPDCKTILRALGPGATLEEMMTACQGVGGPSHKARVLAEAMSQTNSTILMQRSNFKGSKRIVKCFNCGKEGHIARNCRAPRKKGCWKCGKEGHQMKDCTERQANFLGKIWPSHKGRPGNFLQSRPEPTAPPAESFRFEETTPAPKQEPKDREPLTSLRSLFGSDPLSQRENLAFPQGKAREFSSEQTRANSPTRRELQVWGRDNNSLSEAGADRQGTVSFSFPQITLWQRPLVTIKIGGQLKEALLATGADDTVLEEMNLPGRWKPKMIGGIGGFIKVGQYDQIPIEICGHKAIGTVLVGPTPVNIIGRNLLTQIGCTLNFPISPIETVPVKLKPGMDGPKVKQWPLTEEKIKALVEICTEMEKEGKISKIGPENPYNTPIFAIKKKDSTKWRKLVDFRELNKRTQDFWEVQLGIPHPAGLKKKKSVTVLDVGDAYFSVPLDEDFRKYTAFTIPSINNETPGIRYQYNVLPQGWKGSPAIFQSSMTKILEPFRKQNPDIVIYQYMDHLYVGSDLEIGQHRTKIEELRQHLLRWGFTTPDKKHQKEPPFLWMGYELHPDKWTVQPIVLPEKDSWTVNDIQKLVGKLNWASQIYAGIKVKQLCKLLRGTKALTEVVPLTEEAELELAENREILKEPVHGVYYDPSKDLIAEIQKQGQGQWTYQIYQEPFKNLKTGKYARMRGAHTNDVKQLTEAVQKIATESIVIWGKTPKFKLPIQKETWEAWWTEYWQATWIPEWEFVNTPPLVKLWYQLEKEPIVGAETFYVDGAANRETKLGKAGYVTDRGRQKVVSLTDTTNQKTELQAIHLALQDSGLEVNIVTDSQYALGIIQAQPDKSESELVSQIIEQLIKKEKVYLAWVPAHKGIGGNEQVDKLVSRGIRKVLFLDGIDKAQEEHEKYHSNWRAMASEFNLPPIVAKEIVASCDKCQLKGEAIHGQVDCSPGIWQLACTHLEGKVILVAVHVASGYIEAEVIPAETGQETAYFLLKLAGRWPVKTIHTDNGSNFTSATVKAACWWAGIKQEFGIPYNPQSQGVVESINKELKKIIGQVRDQAEHLKTAVQMAVFIHNFKRKGGIGEYSAGERIVDIIASDIQTKELQKQITKIQNFRVYYRDSRDPLWKGPAKLLWKGEGAVVIQDNSDIKVVPRRKAKIIRDYGKQMAGDDCVASRQDED

SEQ ID NO: 29 - protein, 1350 aa, Artificial Sequence
  Synthetic Construct (Mosaic gagpol1 v5)
MGARASVLSGGELDRWEKIRLRPGGKKKYRLKHIVWASRELERFAVNPGLLETSEGCRQILGQLQPSLQTGSEELRSLYNTVATLYCVHQRIEIKDTKEALEKIEEEQNKSKKKAQQAAADTGNSSQVSQNYPIVQNIQGQMVHQAISPRTLNAWVKVVEEKAFSPEVIPMFSALSEGATPQDLNTMLNTVGGHQAAMQMLKETINEEAAEWDRVHPVHAGPIAPGQMREPRGSDIAGTTSTLQEQIGWMTNNPPIPVGEIYKRWIILGLNKIVRMYSPVSILDIRQGPKEPFRDYVDRFYKTLRAEQASQDVKNWMTETLLVQNANPDCKTILKALGPAATLEEMMTACQGVGGPGHKARVLAEAMSQVTNSATIMMQRGNFRNQRKTVKCFNCGKEGHIAKNCRAPRKKGCWKCGKEGHQMKDCTERQANFLGKIWPSNKGRPGNFLQNRPEPTAPPEESFRFGEETTTPSQKQEPIDKEMYPLASLKSLFGNDPSSQMAPISPIETVPVKLKPGMDGPRVKQWPLTEEKIKALTAICEEMEKEGKITKIGPENPYNTPVFAIKKKDSTKWRKLVDFRELNKRTQDFWEVQLGIPHPAGLKKKKSVTVLDVGDAYFSVPLDEGFRKYTAFTIPSTNNETPGIRYQYNVLPQGWKGSPAIFQCSMTRILEPFRAKNPEIVIYQYMDHLYVGSDLEIGQHRAKIEELREHLLKWGFTTPDKKHQKEPPFLWMGYELHPDKWTVQPIQLPEKDSWTVNDIQKLVGKLNWASQIYPGIKVRQLCKLLRGAKALTDIVPLTEEAELELAENREILKEPVHGVYYDPSKDLIAEIQKQGHDQWTYQIYQEPFKNLKTGKYAKMRTAHTNDVKQLTEAVQKIAMESIVIWGKTPKFRLPIQKETWETWWTDYWQATWIPEWEFVNTPPLVKLWYQLEKDPIAGVETFYVDGAANRETKLGKAGYVTDRGRQKIVSLTETTNQKTELQAIYLALQDSGSEVNIVTDSQYALGIIQAQPDKSESELVNQIIEQLIKKERVYLSWVPAHKGIGGNEQVDKLVSSGIRKVLFLDGIDKAQEEHEKYHSNWRAMASDFNLPPVVAKEIVASCDQCQLKGEAMHGQVDCSPGIWQLACTHLEGKIILVAVHVASGYIEAEVIPAETGQETAYFILKLAGRWPVKVIHTDNGSNFTSAAVKAACWWAGIQQEFGIPYNPQSQGVVESMNKELKKIIGQVRDQAEHLKTAVQMAVFIHNFKRKGGIGGYSAGERIIDIIATDIQTKELQKQIIKIQNFRVYYRDSRDPIWKGPAKLLWKGEGAVVIQDNSDIKVVPRRKVKIIKDYGKQMAGADCVAGRQDED

SEQ ID NO: 30 - protein, 1341 aa, Artificial Sequence
  Synthetic Construct (Mosaic gagpol2 v5)
MGARASILRGGKLDKWEKIRLRPGGKKHYMLKHLVWASRELERFALNPGLLETSEGCKQIIKQLQPALQTGTEELRSLFNTVATLYCVHAEIEVRDTKEALDKIEEEQNKSQQKTQQAKEADGKVSQNYPIVQNLQGQMVHQPISPRTLNAWVKVIEEKAFSPEVIPMFTALSEGATPQDLNTMLNTVGGHQAAMQMLKDTINEEAAEWDRLHPVHAGPVAPGQMREPRGSDIAGTTSNLQEQIAWMTSNPPIPVGDIYKRWIILGLNKIVRMYSPTSILDIKQGPKEPFRDYVDRFFKTLRAEQATQDVKNWMTDTLLVQNANPDCKTILRALGPGATLEEMMTACQGVGGPSHKARVLAEAMSQTNSTILMQRSNFKGSKRIVKCFNCGKEGHIARNCRAPRKKGCWKCGKEGHQMKDCTERQANFLGKIWPSHKGRPGNFLQSRPEPTAPPAESFRFEETTPAPKQEPKDREPLTSLRSLFGSDPLSQMAPISPIETVPVKLKPGMDGPKVKQWPLTEEKIKALVEICTEMEKEGKISKIGPENPYNTPIFAIKKKDSTKWRKLVDFRELNKRTQDFWEVQLGIPHPAGLKKKKSVTVLDVGDAYFSVPLDEDFRKYTAFTIPSINNETPGIRYQYNVLPQGWKGSPAIFQSSMTKILEPFRKQNPDIVIYQYMDHLYVGSDLEIGQHRTKIEELRQHLLRWGFTTPDKKHQKEPPFLWMGYELHPDKWTVQPIVLPEKDSWTVNDIQKLVGKLNWASQIYAGIKVKQLCKLLRGTKALTEVVPLTEEAELELAENREILKEPVHGVYYDPSKDLIAEIQKQGQGQWTYQIYQEPFKNLKTGKYARMRGAHTNDVKQLTEAVQKIATESIVIWGKTPKFKLPIQKETWEAWWTEYWQATWIPEWEFVNTPPLVKLWYQLEKEPIVGAETFYVDGAANRETKLGKAGYVTDRGRQKVVSLTDTTNQKTELQAIHLALQDSGLEVNIVTDSQYALGIIQAQPDKSESELVSQIIEQLIKKEKVYLAWVPAHKGIGGNEQVDKLVSRGIRKVLFLDGIDKAQEEHEKYHSNWRAMASEFNLPPIVAKEIVASCDKCQLKGEAIHGQVDCSPGIWQLACTHLEGKVILVAVHVASGYIEAEVIPAETGQETAYFLLKLAGRWPVKTIHTDNGSNFTSATVKAACWWAGIKQEFGIPYNPQSQGVVESINKELKKIIGQVRDQAEHLKTAVQMAVFIHNFKRKGGIGEYSAGERIVDIIASDIQTKELQKQITKIQNFRVYYRDSRDPLWKGPAKLLWKGEGAVVIQDNSDIKVVPRRKAKIIRDYGKQMAGDDCVASRQDED

SEQ ID NO: 31 - protein, 1556 aa, Artificial Sequence
  Synthetic Construct (Mosaic gagpolnef1)
MGARASVLSGGELDRWEKIRLRPGGKKKYRLKHIVWASRELERFAVNPGLLETSEGCRQILGQLQPSLQTGSEELRSLYNTVATLYCVHQRIEIKDTKEALEKIEEEQNKSKKKAQQAAADTGNSSQVSQNYPIVQNIQGQMVHQAISPRTLNAWVKVVEEKAFSPEVIPMFSALSEGATPQDLNTMLNTVGGHQAAMQMLKETINEEAAEWDRVHPVHAGPIAPGQMREPRGSDIAGTTSTLQEQIGWMTNNPPIPVGEIYKRWIILGLNKIVRMYSPVSILDIRQGPKEPFRDYVDRFYKTLRAEQASQDVKNWMTETLLVQNANPDCKTILKALGPAATLEEMMTACQGVGGPGHKARVLAEAMSQVTNSATIMMQRGNFRNQRKTVKCFNCGKEGHIAKNCRAPRKKGCWKCGKEGHQMKDCTERQANFLGKIWPSNKGRPGNFLQNRPEPTAPPEESFRFGEETTTPSQKQEPIDKEMYPLASLKSLFGNDPSSQMAPISPIETVPVKLKPGMDGPRVKQWPLTEEKIKALTAICEEMEKEGKITKIGPENPYNTPVFAIKKKDSTKWRKLVDFRELNKRTQDFWEVQLGIPHPAGLKKKKSVTVLAVGDAYFSVPLDEGFRKYTAFTIPSTNNETPGIRYQYNVLPQGWKGSPAIFQCSMTRILEPFRAKNPEIVIYQYMAALYVGSDLEIGQHRAKIEELREHLLKWGFTTPDKKHQKEPPFLWMGYELHPDKWTVQPIQLPEKDSWTVNDIQKLVGKLNWASQIYPGIKVRQLCKLLRGAKALTDIVPLTEEAELELAENREILKEPVHGVYYDPSKDLIAEIQKQGHDQWTYQIYQEPFKNLKTGKYAKMRTAHTNDVKQLTEAVQKIAMESIVIWGKTPKFRLPIQKETWETWWTDYWQATWIPEWEFVNTPPLVKLWYQLEKDPIAGVETFYVAGAANRETKLGKAGYVTDRGRQKIVSLTETTNQKTALQAIYLALQDSGSEVNIVTASQYALGIIQAQPDKSESELVNQIIEQLIKKERVYLSWVPAHKGIGGNEQVDKLVSSGIRKVLFLDGIDKAQEEHEKYHSNWRAMASDFNLPPVVAKEIVASCDQCQLKGEAMHGQVDCSPGIWQLACTHLEGKIILVAVHVASGYIEAEVIPAETGQETAYFILKLAGRWPVKVIHTANGSNFTSAAVKAACWWAGIQQEFGIPYNPQSQGVVASMNKELKKIIGQVRDQAEHLKTAVQMAVFIHNFKRKGGIGGYSAGERIIDIIATDIQTKELQKQIIKIQNFRVYYRDSRDPIWKGPAKLLWKGEGAVVIQDNSDIKVVPRRKVKIIKDYGKQMAGADCVAGRQDEDMAGKWSKSSVVGWPAIRERMRRAEPAADGVGAVSRDLEKHGAITSSNTAANNADCAWLEAQEEEEVGFPVRPQVPLRPMTYKGALDLSHFLKEKGGLEGLIYSQKRQDILDLWVYHTQGYFPDWQNYTPGPGIRYPLTFGWCFKLVPVEPEKIEEANEGENNSLLHPMSQHGMDDPEKEVLMWKFDSRLAFHHMARELHPEYYKDC

SEQ ID NO: 32 - protein, 1547 aa, Artificial Sequence
  Synthetic Construct (Mosaic gagpolnef2)
MGARASILRGGKLDKWEKIRLRPGGKKHYMLKHLVWASRELERFALNPGLLETSEGCKQIIKQLQPALQTGTEELRSLFNTVATLYCVHAEIEVRDTKEALDKIEEEQNKSQQKTQQAKEADGKVSQNYPIVQNLQGQMVHQPISPRTLNAWVKVIEEKAFSPEVIPMFTALSEGATPQDLNTMLNTVGGHQAAMQMLKDTINEEAAEWDRLHPVHAGPVAPGQMREPRGSDIAGTTSNLQEQIAWMTSNPPIPVGDIYKRWIILGLNKIVRMYSPTSILDIKQGPKEPFRDYVDRFFKTLRAEQATQDVKNWMTDTLLVQNANPDCKTILRALGPGATLEEMMTACQGVGGPSHKARVLAEAMSQTNSTILMQRSNFKGSKRIVKCFNCGKEGHIARNCRAPRKKGCWKCGKEGHQMKDCTERQANFLGKIWPSHKGRPGNFLQSRPEPTAPPAESFRFEETTPAPKQEPKDREPLTSLRSLFGSDPLSQMAPISPIETVPVKLKPGMDGPKVKQWPLTEEKIKALVEICTEMEKEGKISKIGPENPYNTPIFAIKKKDSTKWRKLVDFRELNKRTQDFWEVQLGIPHPAGLKKKKSVTVLAVGDAYFSVPLDEDFRKYTAFTIPSINNETPGIRYQYNVLPQGWKGSPAIFQSSMTKILEPFRKQNPDIVIYQYMAALYVGSDLEIGQHRTKIEELRQHLLRWGFTTPDKKHQKEPPFLWMGYELHPDKWTVQPIVLPEKDSWTVNDIQKLVGKLNWASQIYAGIKVKQLCKLLRGTKALTEVVPLTEEAELELAENREILKEPVHGVYYDPSKDLIAEIQKQGQGQWTYQIYQEPFKNLKTGKYARMRGAHTNDVKQLTEAVQKIATESIVIWGKTPKFKLPIQKETWEAWWTEYWQATWIPEWEFVNTPPLVKLWYQLEKEPIVGAETFYVAGAANRETKLGKAGYVTDRGRQKVVSLTDTTNQKTALQAIHLALQDSGLEVNIVTASQYALGIIQAQPDKSESELVSQIIEQLIKKEKVYLAWVPAHKGIGGNEQVDKLVSRGIRKVLFLDGIDKAQEEHEKYHSNWRAMASEFNLPPIVAKEIVASCDKCQLKGEAIHGQVDCSPGIWQLACTHLEGKVILVAVHVASGYIEAEVIPAETGQETAYFLLKLAGRWPVKTIHTANGSNFTSATVKAACWWAGIKQEFGIPYNPQSQGVVASINKELKKIIGQVRDQAEHLKTAVQMAVFIHNFKRKGGIGEYSAGERIVDIIASDIQTKELQKQITKIQNFRVYYRDSRDPLWKGPAKLLWKGEGAVVIQDNSDIKVVPRRKAKIIRDYGKQMAGDDCVASRQDEDMAGKWSKSSIVGWPAVRERIRRAEPAAEGVGAASQDLDKYGALTSSNTAATNADCAWLEAQEDEEVGFPVKPQVPLRPMTYKAAFDLSFFLKEKGGLDGLIYSKKRQEILDLWVYNTQGFFPDWQNYTPGPGVRYPLTFGWCFKLVPVDPREVEEANKGENNCLLHPMNLHGMDDPEREVLVWRFDSRLAFHHMAREKHPEYYKNC